European Patent Application EP 4 585 591 A1, published July 16, 2025. Title: 脂質ナノ粒子. Applicant: 国立大学法人九州大学. The sequence listing filed with the application follows.

SEQUENCE LISTING (14 sequences)

SEQ ID NO: 1 - DNA, 23 bp, synthetic construct
  source 1..23: mol_type = other DNA
cttttcttacgatggtcgttgga

SEQ ID NO: 2 - DNA, 21 bp, synthetic construct
  source 1..21: mol_type = other DNA
tgaggctataagttgtgggga

SEQ ID NO: 3 - DNA, 23 bp, synthetic construct
  source 1..23: mol_type = other DNA
ttctctgtaccatgacactctgc

SEQ ID NO: 4 - DNA, 21 bp, synthetic construct
  source 1..21: mol_type = other DNA
cgtggaatcttccggctgtag

SEQ ID NO: 5 - DNA, 21 bp, synthetic construct
  source 1..21: mol_type = other DNA
aggtccctatggtgccaatgt

SEQ ID NO: 6 - DNA, 20 bp, synthetic construct
  source 1..20: mol_type = other DNA
cggcaggattttgaggtcca

SEQ ID NO: 7 - DNA, 20 bp, synthetic construct
  source 1..20: mol_type = other DNA
gaagatctggcaccacacct

SEQ ID NO: 8 - DNA, 20 bp, synthetic construct
  source 1..20: mol_type = other DNA
tggtacgaccagaggcatac

SEQ ID NO: 9 - RNA, 21 nt, synthetic construct
  source 1..21: mol_type = other RNA
tctccaaagtttgctctaatt

SEQ ID NO: 10 - RNA, 20 nt, synthetic construct
  source 1..20: mol_type = other RNA
ttagacaaactttggagact

SEQ ID NO: 11 - RNA, 64 nt, synthetic construct
  source 1..64: mol_type = other RNA
tgctgattacttggcgagagctcctagttttggccactgactgactaggagctcgccaagtaat

SEQ ID NO: 12 - RNA, 64 nt, synthetic construct
  source 1..64: mol_type = other RNA
cctgattacttggcgagctcctagtcagtcagtggccaaaactaggagctctcgccaagtaatc

SEQ ID NO: 13 - RNA, 20 nt, synthetic construct
  source 1..20: mol_type = other RNA
tcgaggtggacatcacctac

SEQ ID NO: 14 - RNA, 20 nt, synthetic construct
  source 1..20: mol_type = other RNA
aagaactgcaggctgttctc